European Patent Specification EP 3 330 349 B1, published June 19, 2024. Title: CLEANING COMPOSITIONS INCLUDING ENZYMES. Applicant: P&G. The sequence listing filed with the application follows.

SEQUENCE LISTING (26 sequences)

SEQ ID NO: 1 - protein, 412 aa, Pseudomonas aeruginosa
EIQVLKAPRAVVWKDFLGVNAQFLWFSPERYNKQIDRLQDLGLEWVRLDLHWDRLETAEDQYQLASLDQLVKDLEARQLKSVFYLVGSARFITTAPFYSPFQDQYPPRDPEVFARRMAMLSQRYPSVAAWQVWNEPNLIGFWRPKADPEGYAKLLQASTIALRMVDPEKPVVSAGMAFFSEMPDGRTMFDALGHLGVESLGTIATYHPYTQLPEGNYPWNLDFVSHANQINRALRNAGVPAIWSTEWGWSAYKGPKELQDIIGVEGQADYVLRRLALMSALDYDRIFLFTLSDLDQRASVRDRDYGLLDLDANPKPVYLALQRFLKVTGPKLRPADPPVTEDLPDGSFSIGWTREDGRNVWLFWSARGGNVRLPKLKEATLHDPLSGKVTPLSGSDGLEVPVKSSLQMLVWE

SEQ ID NO: 2 - protein, 480 aa, B. licheniformis
ANLNGTLMQYFEWYMPNDGQHWRRLQNDSAYLAEHGITAVWIPPAYKGTSQADVGYGAYDLYDLGEFHQKGTVRTKYGTKGELQSAIKSLHSRDINVYGDWINHKGGADATEDVTAVEVDPADRNRVISGEHLIKAWTHFHFPGRGSTYSDFKWHWYHFDGTDWDESRKLNRIYKFQGKAWDWEVSNENGNYDYLMYADIDYDHPDVAAEIKRWGTWYANELQLDGFRLDAVKHIKFSFLRDWVNHVREKTGKEMFTVAEYWQNDLGALENYLNKTNFNHSVFDVPLHYQFHAASTQGGGYDMRKLLNGTWSKHPLKSVTFVDNHDTQPGQSLESTVQTWFKPLAYAFILTRESGYPQVFYGDMYGTKGDSQREIPALKHKIEPILKARKQYAYGAQHDYFDHHDIVGWTREGDSSVANSGLAALITDGPGGAKRMYVGRQNAGETWHDITGNRSEPWINSEGWGEFHVNGGSVSIYVQR

SEQ ID NO: 3 - protein, 485 aa, Bacillus sp.
HHNGTNGTMMQYFEWYLPNDGNHWNRLRSDASNLKDKGISAVWIPPAWKGASQNDVGYGAYDLYDLGEFNQKGTIRTKYGTRNQLQAAVNALKSNGIQVYGDVVMNHKGGADATEMVRAVEVNPNNRNQEVSGEYTIEAWTKFDFPGRGNTHSNFKWRWYHFDGVDWDQSRKLNNRIYKFRGDGKGWDWEVDTENGNYDYLMYADIDMDHPEVVNELRNWGVWYTNTLGLDGFRIDAVKHIKYSFTRDWINHVRSATGKNMFAVAEFWKNDLGAIENYLNKTNWNHSVFDVPLHYNLYNASKSGGNYDMRQIFNGTVVQRHPMHAVTFVDNHDSQPEEALESFVEEWFKPLAYALTLTREQGYPSVFYGDYYGIPTHGVPAMKSKIDPILEARQKYAYGRQNDYLDHHNIIGWTREGNTAHPNSGLATIMSDGAGGNKWMFVGRNKAGQVWTDITGNRAGTVTINADGWGNFSVNGGSVSIWVNK

SEQ ID NO: 4 - protein, 485 aa, Bacillus sp.
HHNGTNGTMMQYFEWHLPNDGNHWNRLRDDASNLRNRGITAIWIPPAWKGTSQNDVGYGAYDLYDLGEFNQKGTVRTKYGTRSQLESAIHALKNNGVQVYGDVVMNHKGGADATENVLAVEVNPNNRNQEISGDYTIEAWTKFDFPGRGNTYSDFKWRWYHFDGVDWDQSRQFQNRIYKFRGDGKAWDWEVDSENGNYDYLMYADVDMDHPEVVNELRRWGEWYTNTLNLDGFRIDAVKHIKYSFTRDWLTHVRNATGKEMFAVAEFWKNDLGALENYLNKTNWNHSVFDVPLHYNLYNASNSGGNYDMAKLLNGTVVQKHPMHAVTFVDNHDSQPGESLESFVQEWFKPLAYALILTREQGYPSVFYGDYYGIPTHSVPAMKAKIDPILEARQNFAYGTQHDYFDHHNIIGWTREGNTTHPNSGLATIMSDGPGGEKWMYVGQNKAGQVWHDITGNKPGTVTINADGWANFSVNGGSVSIWVKR

SEQ ID NO: 5 - protein, 484 aa, Bacillus sp.
HHNGTNGTMMQYFEWYLPNDGNHWNRLNSDASNLKSKGITAVWIPPAWKGASQNDVGYGAYDLYDLGEFNQKGTVRTKYGTRSQLQAAVTSLKNNGIQVYGDVVMNHKGGADATEMVRAVEVNPNNRNQEVTGEYTIEAWTRFDFPGRGNTHSSFKWRWYHFDGVDWDQSRRLNNRIYKFRGHGKAWDWEVDTENGNYDYLMYADIDMDHPEVVNELRNWGVWYTNTLGLDGFRIDAVKHIKYSFTRDWINHVRSATGKNMFAVAEFWKNDLGAIENYLQKTNWNHSVFDVPLHYNLYNASKSGGNYDMRNIFNGTVVQRHPSHAVTFVDNHDSQPEEALESFVEEWFKPLAYALTLTREQGYPSVFYGDYYGIPTHGVPAMRSKIDPILEARQKYAYGKQNDYLDHHNIGWTREGNTAHPNSGLATIMSDGAGGSKWMFVGRNKAGQVWSDITGNRTGTVTINADGWGNFSVNGGSVSIWVNK

SEQ ID NO: 6 - protein, 515 aa, Geobacillus Stearophermophilus
AAPFNGTMMQYFEWYLPDDGTLWTKVANEANNLSSLGITALWLPPAYKGTSRSDVGYGVYDLYDLGEFNQKGTVRTKYGTKAQYLQAIQAAHAAGMQVYADVVFDHKGGADGTEWVDAVEVNPSDRNQEISGTYQIQAWTKFDFPGRGNTYSSFKWRWYHFDGVDWDESRKLSRIYKFRGIGKAWDWEVDTENGNYDYLMYADLDMDHPEVVTELKNWGKWYVNTTNIDGFRLDAVKHIKFSFFPDWLSYVRSQTGKPLFTVGEYWSYDINKLHNYITKTNGTMSLFDAPLHNKFYTASKSGGAFDMRTLMTNTLMKDQPTLAVTFVDNHDTEPGQALQSWVDPWFKPLAYAFILTRQEGYPCVFYGDYYGIPQYNIPSLKSKIDPLLIARRDYAYGTQHDYLDHSDIIGWTREGVTEKPGSGLAALITDGPGGSKWMYVGKQHAGKVFYDLTGNRSDTVTINSDGWGEFKVNGGSVSVWVPRKTTVSTIARPITTRPWTGEFVRWTEPRLVAWP

SEQ ID NO: 7 - protein, 485 aa, Geobacillus Stearophermophilus
AAPFNGTMMQYFEWYLPDDGTLWTKVANEANNLSSLGITALWLPPAYKGTSRSDVGYGVYDLYDLGEFNQKGTVRTKYGTKAQYLQAIQAAHAAGMQVYADVVFDHKGGADGTEWVDAVEVNPSDRNQEISGTYQIQAWTKFDFPGRGNTYSSFKWRWYHFDGVDWDESRKLSRIYKFRGGKAWDWEVDTENGNYDYLMYADLDMDHPEVVTELKNWGKWYVNTTNIDGFRLDAVKHIKFSFFPDWLSYVRSQTGKPLFTVGEYWSYDINKLHNYITKTNGTMSLFDAPLHNKFYTASKSGGAFDMRTLMTNTLMKDQPTLAVTFVDNHDTEPGQALQSWVDPWFKPLAYAFILTRQEGYPCVFYGDYYGIPQYNIPSLKSKIDPLLIARRDYAYGTQHDYLDHSDIIGWTREGVTEKPGSGLAALITDGPGGSKWMYVGKQHAGKVFYDLTGNRSDTVTINSDGWGEFKVNGGSVSVWVPRKTT

SEQ ID NO: 8 - protein, 483 aa, Artificial
  WO2016091688
HHNGTNGTMMQYFEWYLPNDGNHWNRLNSDASNLKSKGITAVWIPPAWKGASQNDVGYGAYDLYDLGEFNQKGTVRTKYGTRSQLQAAVTSLKNNGIQVYGDVVMNHKGGADATEMVRAVEVNPNNRNQEVTGEYTIEAWTRFDFPGRGNTHSSFKWRWYHFDGVDWDQSRRLNNRIYKFRGKAWDWEVDTENGNYDYLMYADIDMDHPEVVNELRNWGVWYTNTLGLDGFRIDAVKHIKYSFTRDWINHVRSATGKNMFAVAEFWKNDLGAIENYLQKTNWNHSVFDVPLHYNLYNASKSGGNYDMRNIFNGTVVQRHPSHAVTFVDNHDSQPEEALESFVEEWFKPLAYALTLTREQGYPSVFYGDYYGIPTHGVPAMRSKIDPILEARQKYAYGPQHDYLDHPDVIGWTREGDSSHPKSGLATLITDGPGGSKRMYAGLKNAGETWYDITGNRSDTVKIGSDGWGEFHVNDGSVSIYVQK

SEQ ID NO: 9 - protein, 480 aa, Paenibacillus curdlanolyticus
ADNGTIMQYFEWYLPNDGAHWNRLNNDAQNLKNVGITAVWIPPAYKGGSSADVGYGVYDTYDLGEFNQKGTVRTKYGTKSELISAVNNLHAKGIAVYGDVVLNHRMNADATELVDAVEVDPNNRNVETTSTYQIQAWTQYDFPGRGNTYSSFKWRWYHFDGVDWDQSRGLNRIYKLRGDGKDWDWEVDSEYGNYDYLMGADLDFNHPDVVNETKTWGKWFVNTVNLDGVRLDAVKHIKFDFMRDWVNNVRSTTGKNLFAVGEYWHYDVNKLNSYITKTNGTMSLFDVPLHFRFYDASNGGGGYDMRNLLNNTLMSSNPMKAVTFVENHDTQPTQALQSTVQSWFKPLAYATILTREQGYPCVFYGDYYGTSDGKISSYKPIMDKLLNARKVYAYGTQRDYFDHPDIVGWTREGDAAHAGSGLATLITDGPGGSKWMYVGTSKAGQVWTDKTGNRSGTVTIDANGWGNFWVNGGSVSVWAK

SEQ ID NO: 10 - protein, 483 aa, Cytophaga sp.
AATNGTMMQYFEWYVPNDGQQWNRLRTDAPYLSSVGITAVWTPPAYKGTSQADVGYGPYDLYDLGEFNQKGTVRTKYGTKGELKSAVNTLHSNGIQVYGDVVMNHKAGADYTENVTAVEVNPSNRNQETSGEYNIQAWTGFNFPGRGTTYSNFKWQWFHFDGTDWDQSRSLSRIFKFTGKAWDWPVSSENGNYDYLMYADYDYDHPDVVNEMKKWGVWYANEVGLDGYRLDAVKHIKFSFLKDWVDNARAATGKEMFTVGEYWQNDLGALNNYLAKVNYNQSLFDAPLHYNFYAASTGGGYYDMRNILNNTLVASNPTKAVTLVENHDTQPGQSLESTVQPWFKPLAYAFILTRSGGYPSVFYGDMYGTKGTTTREIPALKSKIEPLLKARKDYAYGTQRDYIDNPDVIGWTREGDSTKAKSGLATVITDGPGGSKRMYVGTSNAGEIWYDLTGNNSTKITIGSDGYATFPVNKGSVSVWVQQ

SEQ ID NO: 11 - protein, 618 aa, Bacillus subtilis
LTAPSIKSGTILHAWNWSFNTLKHNMKDIHDAGYTAIQTSPINQVKEGNQGDKSMSNWYWLYQPTSYQIGNRYLGTEQEFKEMCAAAEEYGIKVIVDAVINHTTSDYAAISNEVKSIPNWTHGNTQIKNWSDRWDVTQNSLLGLYDWNTQNTQVQSYLKRFLDRALNDGADGFRFDAAKHIELPDDGSYGSQFWPNITNTSAEFQYGEILQDSASRDAAYANYMDVTASNYGHSIRSALKNRNLGVSNISHYASDVSADKLVTWVESHDTYANDDEESTWMSDDDIRLGWAVIASRSGSTPLFFSRPEGGGNGVRFPGKSQIGDRGSALFEDQAITAVNRFHNVMAGQPEELSNPNGNNQIFMNQRGSHGVVLANAGSSSVSINTATKLPDGRYDNKAGAGSFQVNDGKLTGTINARSVAVLYPDDIAKAPHVFLENYKTGVTHSFNDQLTITLRADANTTKAVYQINNGPETAFKDGDQFTIGKGDPFGKTYTIMLKGTNSDGVTRTEKYSFVKRDPASAKTIGYQNPNHWSQVNAYIYKHDGSRVIELTGSWPGKPMTKNADGIYTLTLPADTDTTNAKVIFNNGSAQVPGQNQPGFDYVLNGLYNDSGLSGSLPH

SEQ ID NO: 12 - protein, 257 aa, Pseudomonas aeruginosa
GGPSSVAFWYAERPPLAELSQFDWVVLEAAHLKPADVGYLKEQGSTPFAYLSVGEFDGDAAAIADSGLARGKSAVRNQAWNSQVMDLAAPSWRAHLLKRAAELRKQGYAGLFLDTLDSFQLQAEERREGQRRALASFLAQLHRQEPGLKLFFNRGFEVLPELPGVASAVAVESIHAGWDAAAGQYREVPQDDRDWLKGHLDALRAQGMPIVAIDYLPPERRDEARALAARLRSEGYVPFVSTPALDYLGVSDVEVQP

SEQ ID NO: 13 - protein, 109 aa, Bacillus licheniformis
ARYDDVLYFPASRYPETGAHISDAIKAGHADVCTIERSGADKRRQESLKGIPTKPGFDRDEWPMAMCEEGGKGASVRYVSSSDNRGAGSWVGNRLNGYADGTRILFIVQ

SEQ ID NO: 14 - protein, 109 aa, Bacillus subtilis
ASSYDKVLYFPLSRYPETGSHIRDAIAEGHPDICTIDDGADKRREESLKGIPTKPGYDRDEWPMAVCEEGGAGADVRYVTPSDNRGAGSWVGNQMSSYPDGTRVLFIVQ

SEQ ID NO: 15 - protein, 109 aa, Bacillus licheniformis
ARYDDILYFPASRYPETGAHISDAIKAGHSDVCTIERSGADKRRQESLKGIPTKPGFDRDEWPMAMCEEGGKGASVRYVSSSDNRGAGSWVGNRLSGFADGTRILFIVQ

SEQ ID NO: 16 - protein, 204 aa, Aspergillus oryzae
KTGSGDSQSDPIKADLEVKGQSALPFDVDCWAILCKGAPNVLQRVNEKTKNSNRDRSGANKGPFKDPQKWGIKALPPKNPSWSAQDFKSPEEYAFASSLQGGTNAILAPVNLASQNSQGGVLNGFYSANKVAQFDPSKPQQTKGTWFQITKFTGAAGPYCKALGSNDKSVCDKNKNIAGDWGFDPAKWAYQYDEKNNKFNYVGK

SEQ ID NO: 17 - protein, 188 aa, Trichoderma harzianum
APAPMPTPPGIPTESSARTQLAGLTVAVAGSGTGYSRDLFPTWDAISGNCNAREYVLKRDGEGVQVNNACESQSGTWISPYDNASFTNASSLDIDHMVPLKNAWISGASSWTTAQREALANDVSRPQLWAVSASANRSKGDRSPDQWKPPLTSFYCTYAKSWIDVKSFYKLTITSAEKTALSSMLDTC

SEQ ID NO: 18 - protein, 463 aa, Streptomyces davawensis
DATIVINPGTRYGTWEGWGTSLAWWGNVFGTRDDFADLFFTTKSVTYNGTSLPGLGLNIARYNLGACSWNAVNGETMVKSPNIPAFKQIEGFWQDWNNEDPTSSAWDWTADATQRAMLVKATQRGAVTELFANSPMWWMCYNHNPSGAADGGNNLQTWNYRQHASHLAAVALYARTNWGVNFATVDPFNEPASSWWTASGTQEGCHLDPAVQAAVLPYMRSELDKRGLTGVRISASDETNYDTARSTWSSFGSATKALVSQVNVHGYQGTGGRRDLLYTDVVTTSGKKLWNSETGDSDGTGLSMARNLCYDFRWLHPTAWCYWQVMDPSTGWAMIAYDANTLQPTTVQPKYYVMAQFSRHIRPGMTILDTGVSFAAAAYDASARRLVLVAVNTSTSPQTFTFDLSRFTTVTGGSGGLVPRWNTVTGGGDMYRAYTNTYVTGKSVSATFAAGSVQTLQVDGVTT

SEQ ID NO: 19 - protein, 464 aa, Streptomyces avermitilis
DATIAVNPSTTYGKWEGWGTSLAWWANVFGARDDFADLFFTTKSVTYNGRTLPGLGLNIARYNLGACSWNSVSGESMVASANIPAFKQIEGYWQDWNNEDPTSSAWKWTADAAQRTMLVKATARGATTELFANSPMWWMCLNHNPSGASGGGNNLQSWNYRQHASHLAAVALYAKSNWGVNFATVDPFNEPSSSWWTATGTQEGCHMDASVQAAVLPYLRSELDRRGLTGTKISASDETSYDLARTTWGSFGSSTKALVNRVNVHGYQGSGGRRDLLYTDVVTTAGKALWNSETGDSDGTGLTLASNLCLDFRWLHPTAWVYWQVMDPSSGWAMIAYDASTLQPGAVQTKYYVMAQFSRHIRAGMTIVDTGVGYAAAAYDATARRLVIVAVNTSTSAQTLTFDLSRFSTVTGGTGGLVRRWNTVTGGGGDLYAAHSDTYLSGKSLSVPFAAGAVQTLEVDGVTV

SEQ ID NO: 20 - protein, 458 aa, Trichoderma harzianum
DTTLSIDPTSNWGTWEGWGVSLAWWAKAFGNRDDLANVFFTRNNQVINGQNLPGLGFNIARYNAGACSTNTYNGSSMVVSSSIKPSRQVDGYWLDWASTDPASSSWNWNVDANQRAMLQKAKANGANIFELFSNSPMWWMCLNHNPSGSGSSDNLQSWNYQNHAVYLANIAQHAQQNWGIQFQSVEAFNEPSSGWGPTGTQEGCHFAVSTMATVIGYLNTELAQRGLSSFISASDETSYDLAISTWQGLGSSAQNAVKRVNVHGYQGGGGRRDTLYSLVSQAGKRLWNSEYGDADASGKSMYTNLLLDFTWLHPTAWVYWQAIDGSGWGLIVGDNDQLTLSSASTKYFVLAQLTRHIRPGMQILTTPDGNTVAAYDSGSQKLVIVAANWGSAQTITFDLTRAKTAGSNGATVPRWSTQTSGGDQYKSYSDTKINNGKFSVSFSTGQVQTFEISGVVLK

SEQ ID NO: 21 - protein, 541 aa, Ascobolus stictoideus
QTYTLEAEAGTLTGVTVMNEIAGFSGTGYVGGWDEDADTVSLTFTSDATKLYDVKIRYSGPYGSKYTRISYNGATGGDISLPETTEWATVNAGQALLNAGSNTIKLHNNWGWYLIDAVILTPSVPRPPHQVTDALVNTNSNAVTKQLMKFLVSKYHKAYITGQQELHAHQWVEKNVGKSPAILGLDFMDYSPSRVEFGTTSQAVEQAIDFDKRGGIVTFAWHWNAPSGLINTPGSEWWRGFYTEHTTFDVAAALQNTTNANYNLLIRDIDAIAVQLKRLQTAGVPVLWRPLHEAEGGWFWWGAKGPEPAKKLYKILYDRLTNYHKLNNLIWVWNSVAKDWYPGDEIVDVLSFDSYPAQPGDHGPVSAQYNALVELGKDKKLIAATEVGTIPDPDLMQLYESYWSFFVTWEGEFIENGVHNSLEFLKKLYNNSFVLNLDTIQGWKNGAGSSTTTVKSTTTTPTTTIKSTTTTPVTTPTTVKTTTTPTTTATTVKSTTTTAGPTPTAVAGRWQQCGGIGFTGPTTCEAGTTCNVLNPYYSQCL

SEQ ID NO: 22 - protein, 526 aa, Chaetomium virescens
PRDPGATARTFEAEDATLAGTNVDTALSGFTGTGYVTGFDQAADKVTFTVDSASTELYDLSIRVAAIYGDKRTSVVLNGGASSEVYFPAGETWTNVAAGQLLLNQGSNTIDIVSNWGWYLIDSITLTPSTPRPAHQINEAPVNAAADKNAKALYSYLRSIYGKKILSGQQELSLSNWIAQQTGKTPALVSVDLMDYSPSRVERGTVGTAVEEAIQHHNRGGIVSVLWHWNAPTGLYDTEEHRWWSGFYTSATDFDVAAALSSTTNANYTLLIRDIDAIAVQLKRLQSAGVPVLFRPLHEAEGGWFWWGAKGPEPAKKLWGILYDRVTNHHQINNLLWVWNSILPEWYPGDATVDILSADVYAQGNGPMSTQYNQLIELGKDKKMIAAAEVGAAPLPDLLQAYEAHWLWFTVWGDSFINNADWNSLDTLKKVYTSDYVLTLDEIQGWQGSTPSATTTSSTTTPSATTTTTTPSTTATTATPSATTTASPVTYAEHWGQCAGKGWTGPTTCRPPYTCKYQNDWYSQCL

SEQ ID NO: 23 - protein, 452 aa, Preussia aemulans
QTVIYQAEQAKLSGVTVEFSIIKQVVGTGYVEGFDESTDSITFTVESTTAALYDLALTYNGPYGDKYTNVVLNNAAGSQVSLPATTAWTTVPAGQVLLNAGANTIQIQNNWGWYLVDSISLKPAATRGAHQITTKPVNKNANSDAKALLKYLGSIYGKKILSGQQDLSSLDWVTKNVGKTPAVLGLDTMDYSESRKSRGAVSTDVDKAIAFAKKGGIVTFCWHWGAPTGLFDSAAQPWYRGFYTDATDFNIETALKDTTNANYTLLMKDIDTIAVQLKKLQDAGVPVIWRPLHEAEGGWFWWGAKGPEPAKKLWKIMYDRLTNQHGLNNLVWTWNSVAPNWYPGDDTVDIVSADTYSQGDHGPISATYNNLLALTNDTKIIAAAEIGSVMEPAQLQAYQADWVYFCVWSGEFIDGGVWNSLDFLKKVYNDPYVLTLDEIQGWKTARGKPRVS

SEQ ID NO: 24 - protein, 312 aa, Yunnania penicillata
APSTTPVNEKATDAAKNLLSYLVEQAANGVTLSGQQDLESAQWVSDNVGKWPAILGIDFMDYSPSRVEYGAVGSTVPDAISYDSDGGIVTFCWHWGSPSGTYNTTDQPWWSNFYTEATAFDIAAAMDDPDSADYNLLVRDIDAISELLLQLQDLDIPILWRPLHEAEGGWFWWGAKGPEACIALYRLMFDRMTNHHGLNNLLWVWNSVDPSWYPGNDVVDIVSADIYADAGDHSPQEETFASLQSLTGDTKLVALGEVGNIPDPASTGGVADWAYWVTWNGDFIKGEDYNPLEYKKEVFSAENIITRDEVDV

SEQ ID NO: 25 - protein, 327 aa, Myrothecium roridum
GTIENRQWLTYNPVDSAATTEARALLRYIQSQYGWRYLSGQQERAEVQWLKSNIGKTPAIQGSDLIDYSPSRVSYGATSTAVEDAIAFDRQGGIVTFTWHWNAPNCLYNSADQPWYFGFYTKATCFNIQAALAQGSNGADYKLLIRDIDAIAVQLKRLRDAKVPILFRPLHEPDGAWFWWGAKGSGPFKQLWDILYDRLTKYHGLHNMLWVCNTEKSDWYPGNNKCDIATTDVYVNAGDHSVQKSHWDALYGVSGGQRILALGEVGVIPDPERQASENVPWAYWMTWNGYFIRDGNYNSRNFLQSTFSNARVVTLDGTSPLGNWKSS

SEQ ID NO: 26 - protein, 361 aa, Aggregatibacter actinomycetemcomitans
NCCVKGNSIYPQKTSTKQTGLMLDIARHFYSPEVIKSFIDTISLSGGNFLHLHFSDHENYAIESHLLNQRAENAVQGKDGIYINPYTGKPFLSYRQLDDIKAYAKAKGIELIPELDSPNHMTAIFKLVQKDRGVKYLQGLKSRQVDDEIDITNADSITFMQSLMSEVIDIFGDTSQHFHIGGDEFGYSVESNHEFITYANKLSYFLEKKGLKTRMWNDGLIKNTFEQINPNIEITYWSYDGDTQDKNEAAERRDMRVSLPELLAKGFTVLNYNSYYLYIVPKASPTFSQDAAFAAKDVIKNWDLGVWDGRNTKNRVQNTHEIAGAALSIWGEDAKALKDETIQKNTKSLLEAVIHKTNGDE